European Patent Application EP 4 549 934 A1, published May 7, 2025. Title: C9 nanopores. Applicant: Adolphe Merkle Institute. The sequence listing filed with the application follows.

SEQUENCE LISTING (1 sequence)

SEQ ID NO: 1 - protein, 506 aa, Homo sapiens
SHIDCRMSPWSEWSQCDPCLRQMFRSRSIEVFGQFNGKRCTDAVGDRRQCVPTEPCEDAEDDCGNDFQCSTGRCIKMRLRCNGDNDCGDFSDEDDCESEPRPPCRDRVVEESELARTAGYGINILGMDPLSTPFDNEFYNGLCNRDRDGNTLTYYRRPWNVASLIYETKGEKNFRTEHYEEQIEAFKSIIQEKTSNFNAAISLKFTPTETNKAEQCCEETASSISLHGKGSFRFSYSKNETYQLFLSYSSKKEKMFLHVKGEIHLGRFVMRNRDVVLTTTFVDDIKALPTTYEKGEYFAFLETYGTHYSSSGSLGGLYELIYVLDKASMKRKGVELKDIKRCLGYHLDVSLAFSEISVGAEFNKDDCVKRGEGRAVNITSENLIDDVVSLIRGGTRKYAFELKEKLLRGTVIDVTDFVNWASSINDAPVLISQKLSPIYNLVPVKMKNAHLKKQNLERAIEDYINEFSVRKCHTCQNGGTVILMDGKCLCACPFKFEGIACEISKQ